European Patent Specification EP 3 653 729 B1, published October 15, 2025. Title: DNA POLYMERASES WITH INCREASED MUTATION SPECIFIC AMPLIFICATION. Applicant: GeneCast Co., Ltd. The sequence listing filed with the application follows.

SEQUENCE LISTING (61 sequences)

SEQ ID NO: 1 - protein, 832 aa, Artificial Sequence [sequence omitted]

SEQ ID NO: 2 - protein, 832 aa, Artificial Sequence
  Taq E507K
MRGMLPLFEPKGRVLLVDGHHLAYRTFHALKGLTTSRGEPVQAVYGFAKSLLKALKEDGDAVIVVFDAKAPSFRHEAYGGYKAGRAPTPEDFPRQLALIKELVDLLGLARLEVPGYEADDVLASLAKKAEKEGYEVRILTADKDLYQLLSDRIHVLHPEGYLITPAWLWEKYGLRPDQWADYRALTGDESDNLPGVKGIGEKTARKLLEEWGSLEALLKNLDRLKPAIREKILAHMDDLKLSWDLAKVRTDLPLEVDFAKRREPDRERLRAFLERLEFGSLLHEFGLLESPKALEEAPWPPPEGAFVGFVLSRKEPMWADLLALAAARGGRVHRAPEPYKALRDLKEARGLLAKDLSVLALREGLGLPPGDDPMLLAYLLDPSNTTPEGVARRYGGEWTEEAGERAALSERLFANLWGRLEGEERLLWLYREVERPLSAVLAHMEATGVRLDVAYLRALSLEVAEEIARLEAEVFRLAGHPFNLNSRDQLERVLFDELGLPAIGKTKKTGKRSTSAAVLEALREAHPIVEKILQYRELTKLKSTYIDPLPDLIHPRTGRLHTRFNQTATATGRLSSSDPNLQNIPVRTPLGQRIRRAFIAEEGWLLVALDYSQIELRVLAHLSGDENLIRVFQEGRDIHTETASWMFGVPREAVDPLMRRAAKTINFGVLYGMSAHRLSQELAIPYEEAQAFIERYFQSFPKVRAWIEKTLEEGRRRGYVETLFGRRRYVPDLEARVKSVREAAERMAFNMPVQGTAADLMKLAMVKLFPRLEEMGARMLLQVHDELVLEAPKERAEAVARLAKEVMEGVYPLAVPLEVEVGIGEDWLSAKE

SEQ ID NO: 3 - protein, 832 aa, Artificial Sequence
  Taq R536K
MRGMLPLFEPKGRVLLVDGHHLAYRTFHALKGLTTSRGEPVQAVYGFAKSLLKALKEDGDAVIVVFDAKAPSFRHEAYGGYKAGRAPTPEDFPRQLALIKELVDLLGLARLEVPGYEADDVLASLAKKAEKEGYEVRILTADKDLYQLLSDRIHVLHPEGYLITPAWLWEKYGLRPDQWADYRALTGDESDNLPGVKGIGEKTARKLLEEWGSLEALLKNLDRLKPAIREKILAHMDDLKLSWDLAKVRTDLPLEVDFAKRREPDRERLRAFLERLEFGSLLHEFGLLESPKALEEAPWPPPEGAFVGFVLSRKEPMWADLLALAAARGGRVHRAPEPYKALRDLKEARGLLAKDLSVLALREGLGLPPGDDPMLLAYLLDPSNTTPEGVARRYGGEWTEEAGERAALSERLFANLWGRLEGEERLLWLYREVERPLSAVLAHMEATGVRLDVAYLRALSLEVAEEIARLEAEVFRLAGHPFNLNSRDQLERVLFDELGLPAIGKTEKTGKRSTSAAVLEALREAHPIVEKILQYKELTKLKSTYIDPLPDLIHPRTGRLHTRFNQTATATGRLSSSDPNLQNIPVRTPLGQRIRRAFIAEEGWLLVALDYSQIELRVLAHLSGDENLIRVFQEGRDIHTETASWMFGVPREAVDPLMRRAAKTINFGVLYGMSAHRLSQELAIPYEEAQAFIERYFQSFPKVRAWIEKTLEEGRRRGYVETLFGRRRYVPDLEARVKSVREAAERMAFNMPVQGTAADLMKLAMVKLFPRLEEMGARMLLQVHDELVLEAPKERAEAVARLAKEVMEGVYPLAVPLEVEVGIGEDWLSAKE

SEQ ID NO: 4 - protein, 832 aa, Artificial Sequence
  Taq R660V
MRGMLPLFEPKGRVLLVDGHHLAYRTFHALKGLTTSRGEPVQAVYGFAKSLLKALKEDGDAVIVVFDAKAPSFRHEAYGGYKAGRAPTPEDFPRQLALIKELVDLLGLARLEVPGYEADDVLASLAKKAEKEGYEVRILTADKDLYQLLSDRIHVLHPEGYLITPAWLWEKYGLRPDQWADYRALTGDESDNLPGVKGIGEKTARKLLEEWGSLEALLKNLDRLKPAIREKILAHMDDLKLSWDLAKVRTDLPLEVDFAKRREPDRERLRAFLERLEFGSLLHEFGLLESPKALEEAPWPPPEGAFVGFVLSRKEPMWADLLALAAARGGRVHRAPEPYKALRDLKEARGLLAKDLSVLALREGLGLPPGDDPMLLAYLLDPSNTTPEGVARRYGGEWTEEAGERAALSERLFANLWGRLEGEERLLWLYREVERPLSAVLAHMEATGVRLDVAYLRALSLEVAEEIARLEAEVFRLAGHPFNLNSRDQLERVLFDELGLPAIGKTEKTGKRSTSAAVLEALREAHPIVEKILQYRELTKLKSTYIDPLPDLIHPRTGRLHTRFNQTATATGRLSSSDPNLQNIPVRTPLGQRIRRAFIAEEGWLLVALDYSQIELRVLAHLSGDENLIRVFQEGRDIHTETASWMFGVPREAVDPLMRVAAKTINFGVLYGMSAHRLSQELAIPYEEAQAFIERYFQSFPKVRAWIEKTLEEGRRRGYVETLFGRRRYVPDLEARVKSVREAAERMAFNMPVQGTAADLMKLAMVKLFPRLEEMGARMLLQVHDELVLEAPKERAEAVARLAKEVMEGVYPLAVPLEVEVGIGEDWLSAKE

SEQ ID NO: 5 - protein, 832 aa, Artificial Sequence
  Taq R536K/R660V
MRGMLPLFEPKGRVLLVDGHHLAYRTFHALKGLTTSRGEPVQAVYGFAKSLLKALKEDGDAVIVVFDAKAPSFRHEAYGGYKAGRAPTPEDFPRQLALIKELVDLLGLARLEVPGYEADDVLASLAKKAEKEGYEVRILTADKDLYQLLSDRIHVLHPEGYLITPAWLWEKYGLRPDQWADYRALTGDESDNLPGVKGIGEKTARKLLEEWGSLEALLKNLDRLKPAIREKILAHMDDLKLSWDLAKVRTDLPLEVDFAKRREPDRERLRAFLERLEFGSLLHEFGLLESPKALEEAPWPPPEGAFVGFVLSRKEPMWADLLALAAARGGRVHRAPEPYKALRDLKEARGLLAKDLSVLALREGLGLPPGDDPMLLAYLLDPSNTTPEGVARRYGGEWTEEAGERAALSERLFANLWGRLEGEERLLWLYREVERPLSAVLAHMEATGVRLDVAYLRALSLEVAEEIARLEAEVFRLAGHPFNLNSRDQLERVLFDELGLPAIGKTEKTGKRSTSAAVLEALREAHPIVEKILQYKELTKLKSTYIDPLPDLIHPRTGRLHTRFNQTATATGRLSSSDPNLQNIPVRTPLGQRIRRAFIAEEGWLLVALDYSQIELRVLAHLSGDENLIRVFQEGRDIHTETASWMFGVPREAVDPLMRVAAKTINFGVLYGMSAHRLSQELAIPYEEAQAFIERYFQSFPKVRAWIEKTLEEGRRRGYVETLFGRRRYVPDLEARVKSVREAAERMAFNMPVQGTAADLMKLAMVKLFPRLEEMGARMLLQVHDELVLEAPKERAEAVARLAKEVMEGVYPLAVPLEVEVGIGEDWLSAKE

SEQ ID NO: 6 - protein, 832 aa, Artificial Sequence
  Taq E507K/R536K
MRGMLPLFEPKGRVLLVDGHHLAYRTFHALKGLTTSRGEPVQAVYGFAKSLLKALKEDGDAVIVVFDAKAPSFRHEAYGGYKAGRAPTPEDFPRQLALIKELVDLLGLARLEVPGYEADDVLASLAKKAEKEGYEVRILTADKDLYQLLSDRIHVLHPEGYLITPAWLWEKYGLRPDQWADYRALTGDESDNLPGVKGIGEKTARKLLEEWGSLEALLKNLDRLKPAIREKILAHMDDLKLSWDLAKVRTDLPLEVDFAKRREPDRERLRAFLERLEFGSLLHEFGLLESPKALEEAPWPPPEGAFVGFVLSRKEPMWADLLALAAARGGRVHRAPEPYKALRDLKEARGLLAKDLSVLALREGLGLPPGDDPMLLAYLLDPSNTTPEGVARRYGGEWTEEAGERAALSERLFANLWGRLEGEERLLWLYREVERPLSAVLAHMEATGVRLDVAYLRALSLEVAEEIARLEAEVFRLAGHPFNLNSRDQLERVLFDELGLPAIGKTKKTGKRSTSAAVLEALREAHPIVEKILQYKELTKLKSTYIDPLPDLIHPRTGRLHTRFNQTATATGRLSSSDPNLQNIPVRTPLGQRIRRAFIAEEGWLLVALDYSQIELRVLAHLSGDENLIRVFQEGRDIHTETASWMFGVPREAVDPLMRRAAKTINFGVLYGMSAHRLSQELAIPYEEAQAFIERYFQSFPKVRAWIEKTLEEGRRRGYVETLFGRRRYVPDLEARVKSVREAAERMAFNMPVQGTAADLMKLAMVKLFPRLEEMGARMLLQVHDELVLEAPKERAEAVARLAKEVMEGVYPLAVPLEVEVGIGEDWLSAKE

SEQ ID NO: 7 - protein, 832 aa, Artificial Sequence
  Taq E507K/R660V
MRGMLPLFEPKGRVLLVDGHHLAYRTFHALKGLTTSRGEPVQAVYGFAKSLLKALKEDGDAVIVVFDAKAPSFRHEAYGGYKAGRAPTPEDFPRQLALIKELVDLLGLARLEVPGYEADDVLASLAKKAEKEGYEVRILTADKDLYQLLSDRIHVLHPEGYLITPAWLWEKYGLRPDQWADYRALTGDESDNLPGVKGIGEKTARKLLEEWGSLEALLKNLDRLKPAIREKILAHMDDLKLSWDLAKVRTDLPLEVDFAKRREPDRERLRAFLERLEFGSLLHEFGLLESPKALEEAPWPPPEGAFVGFVLSRKEPMWADLLALAAARGGRVHRAPEPYKALRDLKEARGLLAKDLSVLALREGLGLPPGDDPMLLAYLLDPSNTTPEGVARRYGGEWTEEAGERAALSERLFANLWGRLEGEERLLWLYREVERPLSAVLAHMEATGVRLDVAYLRALSLEVAEEIARLEAEVFRLAGHPFNLNSRDQLERVLFDELGLPAIGKTKKTGKRSTSAAVLEALREAHPIVEKILQYRELTKLKSTYIDPLPDLIHPRTGRLHTRFNQTATATGRLSSSDPNLQNIPVRTPLGQRIRRAFIAEEGWLLVALDYSQIELRVLAHLSGDENLIRVFQEGRDIHTETASWMFGVPREAVDPLMRVAAKTINFGVLYGMSAHRLSQELAIPYEEAQAFIERYFQSFPKVRAWIEKTLEEGRRRGYVETLFGRRRYVPDLEARVKSVREAAERMAFNMPVQGTAADLMKLAMVKLFPRLEEMGARMLLQVHDELVLEAPKERAEAVARLAKEVMEGVYPLAVPLEVEVGIGEDWLSAKE

SEQ ID NO: 8 - protein, 832 aa, Artificial Sequence
  Taq E507K/R536K/R660V
MRGMLPLFEPKGRVLLVDGHHLAYRTFHALKGLTTSRGEPVQAVYGFAKSLLKALKEDGDAVIVVFDAKAPSFRHEAYGGYKAGRAPTPEDFPRQLALIKELVDLLGLARLEVPGYEADDVLASLAKKAEKEGYEVRILTADKDLYQLLSDRIHVLHPEGYLITPAWLWEKYGLRPDQWADYRALTGDESDNLPGVKGIGEKTARKLLEEWGSLEALLKNLDRLKPAIREKILAHMDDLKLSWDLAKVRTDLPLEVDFAKRREPDRERLRAFLERLEFGSLLHEFGLLESPKALEEAPWPPPEGAFVGFVLSRKEPMWADLLALAAARGGRVHRAPEPYKALRDLKEARGLLAKDLSVLALREGLGLPPGDDPMLLAYLLDPSNTTPEGVARRYGGEWTEEAGERAALSERLFANLWGRLEGEERLLWLYREVERPLSAVLAHMEATGVRLDVAYLRALSLEVAEEIARLEAEVFRLAGHPFNLNSRDQLERVLFDELGLPAIGKEKKTGKRSTSAAVLEALREAHPIVEKILQYKELTKLKSTYIDPLPDLIHPRTGRLHTRFNQTATATGRLSSSDPNLQNIPVRTPLGQRIRRAFIAEEGWLLVALDYSQIELRVLAHLSGDENLIRVFQEGRDIHTETASWMFGVPREAVDPLMRVAAKTINFGVLYGMSAHRLSQELAIPYEEAQAFIERYFQSFPKVRAWIEKTLEEGRRRGYVETLFGRRRYVPDLEARVKSVREAAERMAFNMPVQGTAADLMKLAMVKLFPRLEEMGARMLLQVHDELVLEAPKERAEAVARLAKEVMEGVYPLAVPLEVEVGIGEDWLSAKE

SEQ ID NO: 9 - DNA, 2499 bp, Artificial Sequence
  Thermus aquaticus DNA polymerase (Taq)
atgagggggatgctgcccctctttgagcccaagggccgggtcctcctggtggacggccaccacctggcctaccgcaccttccacgccctgaagggcctcaccaccagccggggggagccggtgcaggcggtctacggcttcgccaagagcctcctcaaggccctcaaggaggacggggacgcggtgatcgtggtctttgacgccaaggccccctccttccgccacgaggcctacggggggtacaaggcgggccgggcccccacgccggaggactttccccggcaactcgccctcatcaaggagctggtggacctcctggggctggcgcgcctcgaggtcccgggctacgaggcggacgacgtcctggccagcctggccaagaaggcggaaaaggagggctacgaggtccgcatcctcaccgccgacaaagacctttaccagctcctttccgaccgcatccacgtcctccaccccgaggggtacctcatcaccccggcctggctttgggaaaagtacggcctgaggcccgaccagtgggccgactaccgggccctgaccggggacgagtccgacaaccttcccggggtcaagggcatcggggagaagacggcgaggaagcttctggaggagtgggggagcctggaagccctcctcaagaacctggaccggctgaagcccgccatccgggagaagatcctggcccacatggacgatctgaagctctcctgggacctggccaaggtgcgcaccgacctgcccctggaggtggacttcgccaaaaggcgggagcccgaccgggagaggcttagggcctttctggagaggcttgagtttggcagcctcctccacgagttcggccttctggaaagccccaaggccctggaggaggccccctggcccccgccggaaggggccttcgtgggctttgtgctttcccgcaaggagcccatgtgggccgatcttctggccctggccgccgccagggggggccgggtccaccgggcccccgagccttataaagccctcagggacctgaaggaggcgcgggggcttctcgccaaagacctgagcgttctggccctgagggaaggccttggcctcccgcccggcgacgaccccatgctcctcgcctacctcctggacccttccaacaccacccccgagggggtggcccggcgctacggcggggagtggacggaggaggcgggggagcgggccgccctttccgagaggctcttcgccaacctgtgggggaggcttgagggggaggagaggctcctttggctttaccgggaggtggagaggcccctttccgctgtcctggcccacatggaggccacgggggtgcgcctggacgtggcctatctcagggccttgtccctggaggtggccgaggagatcgcccgcctcgaggccgaggtcttccgcctggccggccaccccttcaacctcaactcccgggaccagctggaaagggtcctctttgacgagctagggcttcccgccatcggcaagacggagaagaccggcaagcgctccaccagcgccgccgtcctggaggccctccgcgaggcccaccccatcgtggagaagatcctgcagtaccgggagctcaccaagctgaagagcacctacattgaccccttgccggacctcatccaccccaggacgggccgcctccacacccgcttcaaccagacggccacggccacgggcaggctaagtagctccgatcccaacctccagaacatccccgtccgcaccccgcttgggcagaggatccgccgggccttcatcgccgaggaggggtggctattggtggccctggactatagccagatagagctcagggtgctggcccacctctccggcgacgagaacctgatccgggtcttccaggaggggcgggacatccacacggagaccgccagctggatgttcggcgtcccccgggaggccgtggaccccctgatgcgccgggcggccaagaccatcaacttcggggtcctctacggcatgtcggcccaccgcctctcccaggagctagccatcccttacgaggaggcccaggccttcattgagcgctactttcagagcttccccaaggtgcgggcctggattgagaagaccctggaggagggcaggaggcgggggtacgtggagaccctcttcggccgccgccgctacgtgccagacctagaggcccgggtgaagagcgtgcgggaggcggccgagcgcatggccttcaacatgcccgtccagggcaccgccgccgacctcatgaagctggctatggtgaagctcttccccaggctggaggaaatgggggccaggatgctccttcaggtccacgacgagctggtcctcgaggccccaaaagagagggcggaggccgtggcccggctggccaaggaggtcatggagggggtgtatcccctggccgtgcccctggaggtggaggtggggataggggaggactggctctccgccaaggagtga

SEQ ID NO: 10 - DNA, 2499 bp, Artificial Sequence
  Taq E507K
atgagggggatgctgcccctctttgagcccaagggccgggtcctcctggtggacggccaccacctggcctaccgcaccttccacgccctgaagggcctcaccaccagccggggggagccggtgcaggcggtctacggcttcgccaagagcctcctcaaggccctcaaggaggacggggacgcggtgatcgtggtctttgacgccaaggccccctccttccgccacgaggcctacggggggtacaaggcgggccgggcccccacgccggaggactttccccggcaactcgccctcatcaaggagctggtggacctcctggggctggcgcgcctcgaggtcccgggctacgaggcggacgacgtcctggccagcctggccaagaaggcggaaaaggagggctacgaggtccgcatcctcaccgccgacaaagacctttaccagctcctttccgaccgcatccacgtcctccaccccgaggggtacctcatcaccccggcctggctttgggaaaagtacggcctgaggcccgaccagtgggccgactaccgggccctgaccggggacgagtccgacaaccttcccggggtcaagggcatcggggagaagacggcgaggaagcttctggaggagtgggggagcctggaagccctcctcaagaacctggaccggctgaagcccgccatccgggagaagatcctggcccacatggacgatctgaagctctcctgggacctggccaaggtgcgcaccgacctgcccctggaggtggacttcgccaaaaggcgggagcccgaccgggagaggcttagggcctttctggagaggcttgagtttggcagcctcctccacgagttcggccttctggaaagccccaaggccctggaggaggccccctggcccccgccggaaggggccttcgtgggctttgtgctttcccgcaaggagcccatgtgggccgatcttctggccctggccgccgccagggggggccgggtccaccgggcccccgagccttataaagccctcagggacctgaaggaggcgcgggggcttctcgccaaagacctgagcgttctggccctgagggaaggccttggcctcccgcccggcgacgaccccatgctcctcgcctacctcctggacccttccaacaccacccccgagggggtggcccggcgctacggcggggagtggacggaggaggcgggggagcgggccgccctttccgagaggctcttcgccaacctgtgggggaggcttgagggggaggagaggctcctttggctttaccgggaggtggagaggcccctttccgctgtcctggcccacatggaggccacgggggtgcgcctggacgtggcctatctcagggccttgtccctggaggtggccgaggagatcgcccgcctcgaggccgaggtcttccgcctggccggccaccccttcaacctcaactcccgggaccagctggaaagggtcctctttgacgagctagggcttcccgccatcggcaagacgaaaaagaccggcaagcgctccaccagcgccgccgtcctggaggccctccgcgaggcccaccccatcgtggagaagatcctgcagtaccgggagctcaccaagctgaagagcacctacattgaccccttgccggacctcatccaccccaggacgggccgcctccacacccgcttcaaccagacggccacggccacgggcaggctaagtagctccgatcccaacctccagaacatccccgtccgcaccccgcttgggcagaggatccgccgggccttcatcgccgaggaggggtggctattggtggccctggactatagccagatagagctcagggtgctggcccacctctccggcgacgagaacctgatccgggtcttccaggaggggcgggacatccacacggagaccgccagctggatgttcggcgtcccccgggaggccgtggaccccctgatgcgccgggcggccaagaccatcaacttcggggtcctctacggcatgtcggcccaccgcctctcccaggagctagccatcccttacgaggaggcccaggccttcattgagcgctactttcagagcttccccaaggtgcgggcctggattgagaagaccctggaggagggcaggaggcgggggtacgtggagaccctcttcggccgccgccgctacgtgccagacctagaggcccgggtgaagagcgtgcgggaggcggccgagcgcatggccttcaacatgcccgtccagggcaccgccgccgacctcatgaagctggctatggtgaagctcttccccaggctggaggaaatgggggccaggatgctccttcaggtccacgacgagctggtcctcgaggccccaaaagagagggcggaggccgtggcccggctggccaaggaggtcatggagggggtgtatcccctggccgtgcccctggaggtggaggtggggataggggaggactggctctccgccaaggagtga

SEQ ID NO: 11 - DNA, 2499 bp, Artificial Sequence
  Taq R536K
atgagggggatgctgcccctctttgagcccaagggccgggtcctcctggtggacggccaccacctggcctaccgcaccttccacgccctgaagggcctcaccaccagccggggggagccggtgcaggcggtctacggcttcgccaagagcctcctcaaggccctcaaggaggacggggacgcggtgatcgtggtctttgacgccaaggccccctccttccgccacgaggcctacggggggtacaaggcgggccgggcccccacgccggaggactttccccggcaactcgccctcatcaaggagctggtggacctcctggggctggcgcgcctcgaggtcccgggctacgaggcggacgacgtcctggccagcctggccaagaaggcggaaaaggagggctacgaggtccgcatcctcaccgccgacaaagacctttaccagctcctttccgaccgcatccacgtcctccaccccgaggggtacctcatcaccccggcctggctttgggaaaagtacggcctgaggcccgaccagtgggccgactaccgggccctgaccggggacgagtccgacaaccttcccggggtcaagggcatcggggagaagacggcgaggaagcttctggaggagtgggggagcctggaagccctcctcaagaacctggaccggctgaagcccgccatccgggagaagatcctggcccacatggacgatctgaagctctcctgggacctggccaaggtgcgcaccgacctgcccctggaggtggacttcgccaaaaggcgggagcccgaccgggagaggcttagggcctttctggagaggcttgagtttggcagcctcctccacgagttcggccttctggaaagccccaaggccctggaggaggccccctggcccccgccggaaggggccttcgtgggctttgtgctttcccgcaaggagcccatgtgggccgatcttctggccctggccgccgccagggggggccgggtccaccgggcccccgagccttataaagccctcagggacctgaaggaggcgcgggggcttctcgccaaagacctgagcgttctggccctgagggaaggccttggcctcccgcccggcgacgaccccatgctcctcgcctacctcctggacccttccaacaccacccccgagggggtggcccggcgctacggcggggagtggacggaggaggcgggggagcgggccgccctttccgagaggctcttcgccaacctgtgggggaggcttgagggggaggagaggctcctttggctttaccgggaggtggagaggcccctttccgctgtcctggcccacatggaggccacgggggtgcgcctggacgtggcctatctcagggccttgtccctggaggtggccgaggagatcgcccgcctcgaggccgaggtcttccgcctggccggccaccccttcaacctcaactcccgggaccagctggaaagggtcctctttgacgagctagggcttcccgccatcggcaagacggagaagaccggcaagcgctccaccagcgccgccgtcctggaggccctccgcgaggcccaccccatcgtggagaagatcctgcagtacaaggagctcaccaagctgaagagcacctacattgaccccttgccggacctcatccaccccaggacgggccgcctccacacccgcttcaaccagacggccacggccacgggcaggctaagtagctccgatcccaacctccagaacatccccgtccgcaccccgcttgggcagaggatccgccgggccttcatcgccgaggaggggtggctattggtggccctggactatagccagatagagctcagggtgctggcccacctctccggcgacgagaacctgatccgggtcttccaggaggggcgggacatccacacggagaccgccagctggatgttcggcgtcccccgggaggccgtggaccccctgatgcgccgggcggccaagaccatcaacttcggggtcctctacggcatgtcggcccaccgcctctcccaggagctagccatcccttacgaggaggcccaggccttcattgagcgctactttcagagcttccccaaggtgcgggcctggattgagaagaccctggaggagggcaggaggcgggggtacgtggagaccctcttcggccgccgccgctacgtgccagacctagaggcccgggtgaagagcgtgcgggaggcggccgagcgcatggccttcaacatgcccgtccagggcaccgccgccgacctcatgaagctggctatggtgaagctcttccccaggctggaggaaatgggggccaggatgctccttcaggtccacgacgagctggtcctcgaggccccaaaagagagggcggaggccgtggcccggctggccaaggaggtcatggagggggtgtatcccctggccgtgcccctggaggtggaggtggggataggggaggactggctctccgccaaggagtga

SEQ ID NO: 12 - DNA, 2499 bp, Artificial Sequence
  Taq R660V
atgagggggatgctgcccctctttgagcccaagggccgggtcctcctggtggacggccaccacctggcctaccgcaccttccacgccctgaagggcctcaccaccagccggggggagccggtgcaggcggtctacggcttcgccaagagcctcctcaaggccctcaaggaggacggggacgcggtgatcgtggtctttgacgccaaggccccctccttccgccacgaggcctacggggggtacaaggcgggccgggcccccacgccggaggactttccccggcaactcgccctcatcaaggagctggtggacctcctggggctggcgcgcctcgaggtcccgggctacgaggcggacgacgtcctggccagcctggccaagaaggcggaaaaggagggctacgaggtccgcatcctcaccgccgacaaagacctttaccagctcctttccgaccgcatccacgtcctccaccccgaggggtacctcatcaccccggcctggctttgggaaaagtacggcctgaggcccgaccagtgggccgactaccgggccctgaccggggacgagtccgacaaccttcccggggtcaagggcatcggggagaagacggcgaggaagcttctggaggagtgggggagcctggaagccctcctcaagaacctggaccggctgaagcccgccatccgggagaagatcctggcccacatggacgatctgaagctctcctgggacctggccaaggtgcgcaccgacctgcccctggaggtggacttcgccaaaaggcgggagcccgaccgggagaggcttagggcctttctggagaggcttgagtttggcagcctcctccacgagttcggccttctggaaagccccaaggccctggaggaggccccctggcccccgccggaaggggccttcgtgggctttgtgctttcccgcaaggagcccatgtgggccgatcttctggccctggccgccgccagggggggccgggtccaccgggcccccgagccttataaagccctcagggacctgaaggaggcgcgggggcttctcgccaaagacctgagcgttctggccctgagggaaggccttggcctcccgcccggcgacgaccccatgctcctcgcctacctcctggacccttccaacaccacccccgagggggtggcccggcgctacggcggggagtggacggaggaggcgggggagcgggccgccctttccgagaggctcttcgccaacctgtgggggaggcttgagggggaggagaggctcctttggctttaccgggaggtggagaggcccctttccgctgtcctggcccacatggaggccacgggggtgcgcctggacgtggcctatctcagggccttgtccctggaggtggccgaggagatcgcccgcctcgaggccgaggtcttccgcctggccggccaccccttcaacctcaactcccgggaccagctggaaagggtcctctttgacgagctagggcttcccgccatcggcaagacggagaagaccggcaagcgctccaccagcgccgccgtcctggaggccctccgcgaggcccaccccatcgtggagaagatcctgcagtaccgggagctcaccaagctgaagagcacctacattgaccccttgccggacctcatccaccccaggacgggccgcctccacacccgcttcaaccagacggccacggccacgggcaggctaagtagctccgatcccaacctccagaacatccccgtccgcaccccgcttgggcagaggatccgccgggccttcatcgccgaggaggggtggctattggtggccctggactatagccagatagagctcagggtgctggcccacctctccggcgacgagaacctgatccgggtcttccaggaggggcgggacatccacacggagaccgccagctggatgttcggcgtcccccgggaggccgtggaccccctgatgcgcgtggcggccaagaccatcaacttcggggtcctctacggcatgtcggcccaccgcctctcccaggagctagccatcccttacgaggaggcccaggccttcattgagcgctactttcagagcttccccaaggtgcgggcctggattgagaagaccctggaggagggcaggaggcgggggtacgtggagaccctcttcggccgccgccgctacgtgccagacctagaggcccgggtgaagagcgtgcgggaggcggccgagcgcatggccttcaacatgcccgtccagggcaccgccgccgacctcatgaagctggctatggtgaagctcttccccaggctggaggaaatgggggccaggatgctccttcaggtccacgacgagctggtcctcgaggccccaaaagagagggcggaggccgtggcccggctggccaaggaggtcatggagggggtgtatcccctggccgtgcccctggaggtggaggtggggataggggaggactggctctccgccaaggagtga

SEQ ID NO: 13 - DNA, 2499 bp, Artificial Sequence
  Taq R536K/R660V
atgagggggatgctgcccctctttgagcccaagggccgggtcctcctggtggacggccaccacctggcctaccgcaccttccacgccctgaagggcctcaccaccagccggggggagccggtgcaggcggtctacggcttcgccaagagcctcctcaaggccctcaaggaggacggggacgcggtgatcgtggtctttgacgccaaggccccctccttccgccacgaggcctacggggggtacaaggcgggccgggcccccacgccggaggactttccccggcaactcgccctcatcaaggagctggtggacctcctggggctggcgcgcctcgaggtcccgggctacgaggcggacgacgtcctggccagcctggccaagaaggcggaaaaggagggctacgaggtccgcatcctcaccgccgacaaagacctttaccagctcctttccgaccgcatccacgtcctccaccccgaggggtacctcatcaccccggcctggctttgggaaaagtacggcctgaggcccgaccagtgggccgactaccgggccctgaccggggacgagtccgacaaccttcccggggtcaagggcatcggggagaagacggcgaggaagcttctggaggagtgggggagcctggaagccctcctcaagaacctggaccggctgaagcccgccatccgggagaagatcctggcccacatggacgatctgaagctctcctgggacctggccaaggtgcgcaccgacctgcccctggaggtggacttcgccaaaaggcgggagcccgaccgggagaggcttagggcctttctggagaggcttgagtttggcagcctcctccacgagttcggccttctggaaagccccaaggccctggaggaggccccctggcccccgccggaaggggccttcgtgggctttgtgctttcccgcaaggagcccatgtgggccgatcttctggccctggccgccgccagggggggccgggtccaccgggcccccgagccttataaagccctcagggacctgaaggaggcgcgggggcttctcgccaaagacctgagcgttctggccctgagggaaggccttggcctcccgcccggcgacgaccccatgctcctcgcctacctcctggacccttccaacaccacccccgagggggtggcccggcgctacggcggggagtggacggaggaggcgggggagcgggccgccctttccgagaggctcttcgccaacctgtgggggaggcttgagggggaggagaggctcctttggctttaccgggaggtggagaggcccctttccgctgtcctggcccacatggaggccacgggggtgcgcctggacgtggcctatctcagggccttgtccctggaggtggccgaggagatcgcccgcctcgaggccgaggtcttccgcctggccggccaccccttcaacctcaactcccgggaccagctggaaagggtcctctttgacgagctagggcttcccgccatcggcaagacggagaagaccggcaagcgctccaccagcgccgccgtcctggaggccctccgcgaggcccaccccatcgtggagaagatcctgcagtacaaggagctcaccaagctgaagagcacctacattgaccccttgccggacctcatccaccccaggacgggccgcctccacacccgcttcaaccagacggccacggccacgggcaggctaagtagctccgatcccaacctccagaacatccccgtccgcaccccgcttgggcagaggatccgccgggccttcatcgccgaggaggggtggctattggtggccctggactatagccagatagagctcagggtgctggcccacctctccggcgacgagaacctgatccgggtcttccaggaggggcgggacatccacacggagaccgccagctggatgttcggcgtcccccgggaggccgtggaccccctgatgcgcgtggcggccaagaccatcaacttcggggtcctctacggcatgtcggcccaccgcctctcccaggagctagccatcccttacgaggaggcccaggccttcattgagcgctactttcagagcttccccaaggtgcgggcctggattgagaagaccctggaggagggcaggaggcgggggtacgtggagaccctcttcggccgccgccgctacgtgccagacctagaggcccgggtgaagagcgtgcgggaggcggccgagcgcatggccttcaacatgcccgtccagggcaccgccgccgacctcatgaagctggctatggtgaagctcttccccaggctggaggaaatgggggccaggatgctccttcaggtccacgacgagctggtcctcgaggccccaaaagagagggcggaggccgtggcccggctggccaaggaggtcatggagggggtgtatcccctggccgtgcccctggaggtggaggtggggataggggaggactggctctccgccaaggagtga

SEQ ID NO: 14 - DNA, 2499 bp, Artificial Sequence
  Taq E507K/R536
atgagggggatgctgcccctctttgagcccaagggccgggtcctcctggtggacggccaccacctggcctaccgcaccttccacgccctgaagggcctcaccaccagccggggggagccggtgcaggcggtctacggcttcgccaagagcctcctcaaggccctcaaggaggacggggacgcggtgatcgtggtctttgacgccaaggccccctccttccgccacgaggcctacggggggtacaaggcgggccgggcccccacgccggaggactttccccggcaactcgccctcatcaaggagctggtggacctcctggggctggcgcgcctcgaggtcccgggctacgaggcggacgacgtcctggccagcctggccaagaaggcggaaaaggagggctacgaggtccgcatcctcaccgccgacaaagacctttaccagctcctttccgaccgcatccacgtcctccaccccgaggggtacctcatcaccccggcctggctttgggaaaagtacggcctgaggcccgaccagtgggccgactaccgggccctgaccggggacgagtccgacaaccttcccggggtcaagggcatcggggagaagacggcgaggaagcttctggaggagtgggggagcctggaagccctcctcaagaacctggaccggctgaagcccgccatccgggagaagatcctggcccacatggacgatctgaagctctcctgggacctggccaaggtgcgcaccgacctgcccctggaggtggacttcgccaaaaggcgggagcccgaccgggagaggcttagggcctttctggagaggcttgagtttggcagcctcctccacgagttcggccttctggaaagccccaaggccctggaggaggccccctggcccccgccggaaggggccttcgtgggctttgtgctttcccgcaaggagcccatgtgggccgatcttctggccctggccgccgccagggggggccgggtccaccgggcccccgagccttataaagccctcagggacctgaaggaggcgcgggggcttctcgccaaagacctgagcgttctggccctgagggaaggccttggcctcccgcccggcgacgaccccatgctcctcgcctacctcctggacccttccaacaccacccccgagggggtggcccggcgctacggcggggagtggacggaggaggcgggggagcgggccgccctttccgagaggctcttcgccaacctgtgggggaggcttgagggggaggagaggctcctttggctttaccgggaggtggagaggcccctttccgctgtcctggcccacatggaggccacgggggtgcgcctggacgtggcctatctcagggccttgtccctggaggtggccgaggagatcgcccgcctcgaggccgaggtcttccgcctggccggccaccccttcaacctcaactcccgggaccagctggaaagggtcctctttgacgagctagggcttcccgccatcggcaagacgaaaaagaccggcaagcgctccaccagcgccgccgtcctggaggccctccgcgaggcccaccccatcgtggagaagatcctgcagtacaaggagctcaccaagctgaagagcacctacattgaccccttgccggacctcatccaccccaggacgggccgcctccacacccgcttcaaccagacggccacggccacgggcaggctaagtagctccgatcccaacctccagaacatccccgtccgcaccccgcttgggcagaggatccgccgggccttcatcgccgaggaggggtggctattggtggccctggactatagccagatagagctcagggtgctggcccacctctccggcgacgagaacctgatccgggtcttccaggaggggcgggacatccacacggagaccgccagctggatgttcggcgtcccccgggaggccgtggaccccctgatgcgccgggcggccaagaccatcaacttcggggtcctctacggcatgtcggcccaccgcctctcccaggagctagccatcccttacgaggaggcccaggccttcattgagcgctactttcagagcttccccaaggtgcgggcctggattgagaagaccctggaggagggcaggaggcgggggtacgtggagaccctcttcggccgccgccgctacgtgccagacctagaggcccgggtgaagagcgtgcgggaggcggccgagcgcatggccttcaacatgcccgtccagggcaccgccgccgacctcatgaagctggctatggtgaagctcttccccaggctggaggaaatgggggccaggatgctccttcaggtccacgacgagctggtcctcgaggccccaaaagagagggcggaggccgtggcccggctggccaaggaggtcatggagggggtgtatcccctggccgtgcccctggaggtggaggtggggataggggaggactggctctccgccaaggagtga

SEQ ID NO: 15 - DNA, 2499 bp, Artificial Sequence
  Taq E507K/R660V
atgagggggatgctgcccctctttgagcccaagggccgggtcctcctggtggacggccaccacctggcctaccgcaccttccacgccctgaagggcctcaccaccagccggggggagccggtgcaggcggtctacggcttcgccaagagcctcctcaaggccctcaaggaggacggggacgcggtgatcgtggtctttgacgccaaggccccctccttccgccacgaggcctacggggggtacaaggcgggccgggcccccacgccggaggactttccccggcaactcgccctcatcaaggagctggtggacctcctggggctggcgcgcctcgaggtcccgggctacgaggcggacgacgtcctggccagcctggccaagaaggcggaaaaggagggctacgaggtccgcatcctcaccgccgacaaagacctttaccagctcctttccgaccgcatccacgtcctccaccccgaggggtacctcatcaccccggcctggctttgggaaaagtacggcctgaggcccgaccagtgggccgactaccgggccctgaccggggacgagtccgacaaccttcccggggtcaagggcatcggggagaagacggcgaggaagcttctggaggagtgggggagcctggaagccctcctcaagaacctggaccggctgaagcccgccatccgggagaagatcctggcccacatggacgatctgaagctctcctgggacctggccaaggtgcgcaccgacctgcccctggaggtggacttcgccaaaaggcgggagcccgaccgggagaggcttagggcctttctggagaggcttgagtttggcagcctcctccacgagttcggccttctggaaagccccaaggccctggaggaggccccctggcccccgccggaaggggccttcgtgggctttgtgctttcccgcaaggagcccatgtgggccgatcttctggccctggccgccgccagggggggccgggtccaccgggcccccgagccttataaagccctcagggacctgaaggaggcgcgggggcttctcgccaaagacctgagcgttctggccctgagggaaggccttggcctcccgcccggcgacgaccccatgctcctcgcctacctcctggacccttccaacaccacccccgagggggtggcccggcgctacggcggggagtggacggaggaggcgggggagcgggccgccctttccgagaggctcttcgccaacctgtgggggaggcttgagggggaggagaggctcctttggctttaccgggaggtggagaggcccctttccgctgtcctggcccacatggaggccacgggggtgcgcctggacgtggcctatctcagggccttgtccctggaggtggccgaggagatcgcccgcctcgaggccgaggtcttccgcctggccggccaccccttcaacctcaactcccgggaccagctggaaagggtcctctttgacgagctagggcttcccgccatcggcaagacgaaaaagaccggcaagcgctccaccagcgccgccgtcctggaggccctccgcgaggcccaccccatcgtggagaagatcctgcagtaccgggagctcaccaagctgaagagcacctacattgaccccttgccggacctcatccaccccaggacgggccgcctccacacccgcttcaaccagacggccacggccacgggcaggctaagtagctccgatcccaacctccagaacatccccgtccgcaccccgcttgggcagaggatccgccgggccttcatcgccgaggaggggtggctattggtggccctggactatagccagatagagctcagggtgctggcccacctctccggcgacgagaacctgatccgggtcttccaggaggggcgggacatccacacggagaccgccagctggatgttcggcgtcccccgggaggccgtggaccccctgatgcgcgtggcggccaagaccatcaacttcggggtcctctacggcatgtcggcccaccgcctctcccaggagctagccatcccttacgaggaggcccaggccttcattgagcgctactttcagagcttccccaaggtgcgggcctggattgagaagaccctggaggagggcaggaggcgggggtacgtggagaccctcttcggccgccgccgctacgtgccagacctagaggcccgggtgaagagcgtgcgggaggcggccgagcgcatggccttcaacatgcccgtccagggcaccgccgccgacctcatgaagctggctatggtgaagctcttccccaggctggaggaaatgggggccaggatgctccttcaggtccacgacgagctggtcctcgaggccccaaaagagagggcggaggccgtggcccggctggccaaggaggtcatggagggggtgtatcccctggccgtgcccctggaggtggaggtggggataggggaggactggctctccgccaaggagtga

SEQ ID NO: 16 - DNA, 2499 bp, Artificial Sequence
  Taq E507K/R536K/R660V
atgagggggatgctgcccctctttgagcccaagggccgggtcctcctggtggacggccaccacctggcctaccgcaccttccacgccctgaagggcctcaccaccagccggggggagccggtgcaggcggtctacggcttcgccaagagcctcctcaaggccctcaaggaggacggggacgcggtgatcgtggtctttgacgccaaggccccctccttccgccacgaggcctacggggggtacaaggcgggccgggcccccacgccggaggactttccccggcaactcgccctcatcaaggagctggtggacctcctggggctggcgcgcctcgaggtcccgggctacgaggcggacgacgtcctggccagcctggccaagaaggcggaaaaggagggctacgaggtccgcatcctcaccgccgacaaagacctttaccagctcctttccgaccgcatccacgtcctccaccccgaggggtacctcatcaccccggcctggctttgggaaaagtacggcctgaggcccgaccagtgggccgactaccgggccctgaccggggacgagtccgacaaccttcccggggtcaagggcatcggggagaagacggcgaggaagcttctggaggagtgggggagcctggaagccctcctcaagaacctggaccggctgaagcccgccatccgggagaagatcctggcccacatggacgatctgaagctctcctgggacctggccaaggtgcgcaccgacctgcccctggaggtggacttcgccaaaaggcgggagcccgaccgggagaggcttagggcctttctggagaggcttgagtttggcagcctcctccacgagttcggccttctggaaagccccaaggccctggaggaggccccctggcccccgccggaaggggccttcgtgggctttgtgctttcccgcaaggagcccatgtgggccgatcttctggccctggccgccgccagggggggccgggtccaccgggcccccgagccttataaagccctcagggacctgaaggaggcgcgggggcttctcgccaaagacctgagcgttctggccctgagggaaggccttggcctcccgcccggcgacgaccccatgctcctcgcctacctcctggacccttccaacaccacccccgagggggtggcccggcgctacggcggggagtggacggaggaggcgggggagcgggccgccctttccgagaggctcttcgccaacctgtgggggaggcttgagggggaggagaggctcctttggctttaccgggaggtggagaggcccctttccgctgtcctggcccacatggaggccacgggggtgcgcctggacgtggcctatctcagggccttgtccctggaggtggccgaggagatcgcccgcctcgaggccgaggtcttccgcctggccggccaccccttcaacctcaactcccgggaccagctggaaagggtcctctttgacgagctagggcttcccgccatcggcaagacgaaaaagaccggcaagcgctccaccagcgccgccgtcctggaggccctccgcgaggcccaccccatcgtggagaagatcctgcagtacaaggagctcaccaagctgaagagcacctacattgaccccttgccggacctcatccaccccaggacgggccgcctccacacccgcttcaaccagacggccacggccacgggcaggctaagtagctccgatcccaacctccagaacatccccgtccgcaccccgcttgggcagaggatccgccgggccttcatcgccgaggaggggtggctattggtggccctggactatagccagatagagctcagggtgctggcccacctctccggcgacgagaacctgatccgggtcttccaggaggggcgggacatccacacggagaccgccagctggatgttcggcgtcccccgggaggccgtggaccccctgatgcgcgtggcggccaagaccatcaacttcggggtcctctacggcatgtcggcccaccgcctctcccaggagctagccatcccttacgaggaggcccaggccttcattgagcgctactttcagagcttccccaaggtgcgggcctggattgagaagaccctggaggagggcaggaggcgggggtacgtggagaccctcttcggccgccgccgctacgtgccagacctagaggcccgggtgaagagcgtgcgggaggcggccgagcgcatggccttcaacatgcccgtccagggcaccgccgccgacctcatgaagctggctatggtgaagctcttccccaggctggaggaaatgggggccaggatgctccttcaggtccacgacgagctggtcctcgaggccccaaaagagagggcggaggccgtggcccggctggccaaggaggtcatggagggggtgtatcccctggccgtgcccctggaggtggaggtggggataggggaggactggctctccgccaaggagtga

SEQ ID NO: 17 - DNA, 20 bp, Artificial Sequence
  Eco-forward primer
ggggtacctcatcaccccgg

SEQ ID NO: 18 - DNA, 27 bp, Artificial Sequence
  R536K-reverse primer
cttggtgagctccttgtactgcaggat

SEQ ID NO: 19 - DNA, 27 bp, Artificial Sequence
  R536K-forward primer
atcctgcagtacaaggagctcaccaag

SEQ ID NO: 20 - DNA, 30 bp, Artificial Sequence
  R660V-reverse primer
gatggtcttggccgccacgcgcatcagggg

SEQ ID NO: 21 - DNA, 30 bp, Artificial Sequence
  R660V-forward primer
cccctgatgcgcgtggcggccaagaccatc

SEQ ID NO: 22 - DNA, 32 bp, Artificial Sequence
  Xba-reverse primer
gctctagactatcactccttggcggagagcca

SEQ ID NO: 23 - DNA, 27 bp, Artificial Sequence
  E507K-reverse primer
cttgccggtctttttcgtcttgccgat

SEQ ID NO: 24 - DNA, 27 bp, Artificial Sequence
  E507K-forward primer
atcggcaagacgaaaaagaccggcaag

SEQ ID NO: 25 - DNA, 25 bp, Artificial Sequence
  rs1408799 forward primer
ccagtgttaggttatttctaacttg

SEQ ID NO: 26 - DNA, 19 bp, Artificial Sequence
  rs1408799 reverse_T primer
gctcggagcacatggtcaa

SEQ ID NO: 27 - DNA, 19 bp, Artificial Sequence
  rs1408799 reverse_C primer
gctcggagcacatggtcag

SEQ ID NO: 28 - DNA, 22 bp, Artificial Sequence
  rs1015362 forward primer
tgaagagcaggaaagttcttca

SEQ ID NO: 29 - DNA, 20 bp, Artificial Sequence
  rs1015362 reverse_C primer
actgtgtgtctgaaacagtg

SEQ ID NO: 30 - DNA, 20 bp, Artificial Sequence
  rs1015362 reverse_T primer
actgtgtgtctgaaacagta

SEQ ID NO: 31 - DNA, 26 bp, Artificial Sequence
  rs4911414 forward_G primer
gtaagtctttgctgagaaattcattg

SEQ ID NO: 32 - DNA, 26 bp, Artificial Sequence
  rs4911414 forward_T primer
gtaagtctttgctgagaaattcattt

SEQ ID NO: 33 - DNA, 23 bp, Artificial Sequence
  rs4911414 reverse primer
agtatccagggttaatgtgaaag

SEQ ID NO: 34 - DNA, 25 bp, Artificial Sequence
  1408799-FAM probe
agatatttgtaaggtattctggcct

SEQ ID NO: 35 - DNA, 24 bp, Artificial Sequence
  1015362-HEX probe
tgctgaacaaatagtcccgaccag

SEQ ID NO: 36 - DNA, 24 bp, Artificial Sequence
  4911414-Texas Red probe
tttctctagttgcctttaagattt

SEQ ID NO: 37 - protein, 832 aa, Artificial Sequence
  Taq E507K/R536K/R587I/R660V
MRGMLPLFEPKGRVLLVDGHHLAYRTFHALKGLTTSRGEPVQAVYGFAKSLLKALKEDGDAVIVVFDAKAPSFRHEAYGGYKAGRAPTPEDFPRQLALIKELVDLLGLARLEVPGYEADDVLASLAKKAEKEGYEVRILTADKDLYQLLSDRIHVLHPEGYLITPAWLWEKYGLRPDQWADYRALTGDESDNLPGVKGIGEKTARKLLEEWGSLEALLKNLDRLKPAIREKILAHMDDLKLSWDLAKVRTDLPLEVDFAKRREPDRERLRAFLERLEFGSLLHEFGLLESPKALEEAPWPPPEGAFVGFVLSRKEPMWADLLALAAARGGRVHRAPEPYKALRDLKEARGLLAKDLSVLALREGLGLPPGDDPMLLAYLLDPSNTTPEGVARRYGGEWTEEAGERAALSERLFANLWGRLEGEERLLWLYREVERPLSAVLAHMEATGVRLDVAYLRALSLEVAEEIARLEAEVFRLAGHPFNLNSRDQLERVLFDELGLPAIGKEKKTGKRSTSAAVLEALREAHPIVEKILQYKELTKLKSTYIDPLPDLIHPRTGRLHTRFNQTATATGRLSSSDPNLQNIPVITPLGQRIRRAFIAEEGWLLVALDYSQIELRVLAHLSGDENLIRVFQEGRDIHTETASWMFGVPREAVDPLMRVAAKTINFGVLYGMSAHRLSQELAIPYEEAQAFIERYFQSFPKVRAWIEKTLEEGRRRGYVETLFGRRRYVPDLEARVKSVREAAERMAFNMPVQGTAADLMKLAMVKLFPRLEEMGARMLLQVHDELVLEAPKERAEAVARLAKEVMEGVYPLAVPLEVEVGIGEDWLSAKE

SEQ ID NO: 38 - DNA, 2499 bp, Artificial Sequence
  Taq E507K/R536K/R587I/R660V
atgagggggatgctgcccctctttgagcccaagggccgggtcctcctggtggacggccaccacctggcctaccgcaccttccacgccctgaagggcctcaccaccagccggggggagccggtgcaggcggtctacggcttcgccaagagcctcctcaaggccctcaaggaggacggggacgcggtgatcgtggtctttgacgccaaggccccctccttccgccacgaggcctacggggggtacaaggcgggccgggcccccacgccggaggactttccccggcaactcgccctcatcaaggagctggtggacctcctggggctggcgcgcctcgaggtcccgggctacgaggcggacgacgtcctggccagcctggccaagaaggcggaaaaggagggctacgaggtccgcatcctcaccgccgacaaagacctttaccagctcctttccgaccgcatccacgtcctccaccccgaggggtacctcatcaccccggcctggctttgggaaaagtacggcctgaggcccgaccagtgggccgactaccgggccctgaccggggacgagtccgacaaccttcccggggtcaagggcatcggggagaagacggcgaggaagcttctggaggagtgggggagcctggaagccctcctcaagaacctggaccggctgaagcccgccatccgggagaagatcctggcccacatggacgatctgaagctctcctgggacctggccaaggtgcgcaccgacctgcccctggaggtggacttcgccaaaaggcgggagcccgaccgggagaggcttagggcctttctggagaggcttgagtttggcagcctcctccacgagttcggccttctggaaagccccaaggccctggaggaggccccctggcccccgccggaaggggccttcgtgggctttgtgctttcccgcaaggagcccatgtgggccgatcttctggccctggccgccgccagggggggccgggtccaccgggcccccgagccttataaagccctcagggacctgaaggaggcgcgggggcttctcgccaaagacctgagcgttctggccctgagggaaggccttggcctcccgcccggcgacgaccccatgctcctcgcctacctcctggacccttccaacaccacccccgagggggtggcccggcgctacggcggggagtggacggaggaggcgggggagcgggccgccctttccgagaggctcttcgccaacctgtgggggaggcttgagggggaggagaggctcctttggctttaccgggaggtggagaggcccctttccgctgtcctggcccacatggaggccacgggggtgcgcctggacgtggcctatctcagggccttgtccctggaggtggccgaggagatcgcccgcctcgaggccgaggtcttccgcctggccggccaccccttcaacctcaactcccgggaccagctggaaagggtcctctttgacgagctagggcttcccgccatcggcaagacgaaaaagaccggcaagcgctccaccagcgccgccgtcctggaggccctccgcgaggcccaccccatcgtggagaagatcctgcagtacaaggagctcaccaagctgaagagcacctacattgaccccttgccggacctcatccaccccaggacgggccgcctccacacccgcttcaaccagacggccacggccacgggcaggctaagtagctccgatcccaacctccagaacatccccgtcatcaccccgcttgggcagaggatccgccgggccttcatcgccgaggaggggtggctattggtggccctggactatagccagatagagctcagggtgctggcccacctctccggcgacgagaacctgatccgggtcttccaggaggggcgggacatccacacggagaccgccagctggatgttcggcgtcccccgggaggccgtggaccccctgatgcgcgtggcggccaagaccatcaacttcggggtcctctacggcatgtcggcccaccgcctctcccaggagctagccatcccttacgaggaggcccaggccttcattgagcgctactttcagagcttccccaaggtgcgggcctggattgagaagaccctggaggagggcaggaggcgggggtacgtggagaccctcttcggccgccgccgctacgtgccagacctagaggcccgggtgaagagcgtgcgggaggcggccgagcgcatggccttcaacatgcccgtccagggcaccgccgccgacctcatgaagctggctatggtgaagctcttccccaggctggaggaaatgggggccaggatgctccttcaggtccacgacgagctggtcctcgaggccccaaaagagagggcggaggccgtggcccggctggccaaggaggtcatggagggggtgtatcccctggccgtgcccctggaggtggaggtggggataggggaggactggctctccgccaaggagtga

SEQ ID NO: 39 - DNA, 36 bp, Artificial Sequence
  Kpn-forward primer
tccaccccgaggggtacctcatcaccccggcctggc

SEQ ID NO: 40 - DNA, 27 bp, Artificial Sequence
  -forward primer
cccaagcggggtgatgacggggatgtt

SEQ ID NO: 41 - DNA, 27 bp, Artificial Sequence
  R587I-forward primer
aacatccccgtcatcaccccgcttggg

SEQ ID NO: 42 - DNA, 37 bp, Artificial Sequence
  Xba-reverse primer
ctgcaggtcgactctagactatcactccttggcggag

SEQ ID NO: 43 - DNA, 24 bp, Artificial Sequence
  KRAS Q61H forward_Q primer(24mer)
gatattctcgacacagcaggtcaa

SEQ ID NO: 44 - DNA, 24 bp, Artificial Sequence
  KRAS Q61H forward_H primer(24mer)
gatattctcgacacagcaggtcac

SEQ ID NO: 45 - DNA, 20 bp, Artificial Sequence
  KRAS Q61H reverse primer
acaaagaaagccctccccag

SEQ ID NO: 46 - DNA, 25 bp, Artificial Sequence
  KRAS Q61H FAM probe
tgcaatgagggaccagtacatgagg

SEQ ID NO: 47 - DNA, 18 bp, Artificial Sequence
  KRAS Q61H forward_Q primer(18mer)
ctcgacacagcaggtcaa

SEQ ID NO: 48 - DNA, 18 bp, Artificial Sequence
  KRAS Q61H forward_H primer(18mer)
ctcgacacagcaggtcac

SEQ ID NO: 49 - DNA, 20 bp, Artificial Sequence
  KRAS Q61H reverse primer
acaaagaaagccctccccag

SEQ ID NO: 50 - DNA, 21 bp, Artificial Sequence
  KRAS G13D forward primer
ataaggcctgctgaaaatgac

SEQ ID NO: 51 - DNA, 17 bp, Artificial Sequence
  KRAS G13D reverse_G primer(17mer)
ggcactcttgcctacgc

SEQ ID NO: 52 - DNA, 17 bp, Artificial Sequence
  KRAS G13D reverse_D primer(17mer)
ggcactcttgcctacgt

SEQ ID NO: 53 - DNA, 30 bp, Artificial Sequence
  G1213_R FAM
agctccaactaccacaagtttatattcagt

SEQ ID NO: 54 - DNA, 23 bp, Artificial Sequence
  KRAS G12S forward_G primer(23mer)
taaacttgtggtagttggagctg

SEQ ID NO: 55 - DNA, 23 bp, Artificial Sequence
  KRAS G12S forward_S primer(23mer)
taaacttgtggtagttggagcta

SEQ ID NO: 56 - DNA, 28 bp, Artificial Sequence
  KRAS G12S reverse primer
catattcgtccacaaaatgattctgaat

SEQ ID NO: 57 - DNA, 25 bp, Artificial Sequence
  G1213_F FAM probe
agctgtatcgtcaaggcactcttgc

SEQ ID NO: 58 - DNA, 20 bp, Artificial Sequence
  EGFR L858R forward primer
acctggcagccaggaacgta

SEQ ID NO: 59 - DNA, 19 bp, Artificial Sequence
  EGFR L858R reverse_L primer
gcacccagcagtttggcca

SEQ ID NO: 60 - DNA, 19 bp, Artificial Sequence
  EGFR L858R reverse_R primer
gcacccagcagtttggccc

SEQ ID NO: 61 - DNA, 28 bp, Artificial Sequence
  L858R FAM_R probe
cagcatgtcaagatcacagattttgggc